European Patent Specification EP 4 013 453 B1, published March 4, 2026. Title: Hydrophobic Peptide Salts for Extended  Release Compositions. Applicant: Biomarin Pharmaceutical Inc. The sequence listing filed with the application follows.

SEQUENCE LISTING (68 sequences)

SEQ ID NO: 1 - protein, 39 aa, Artificial Sequence
  Synthetic Polypeptide
PGQEHPNARKYKGANKKGLSKGCFGLKLDRIGSMSGLGC

SEQ ID NO: 2 - protein, 38 aa, Artificial Sequence
  Synthetic Polypeptide
LQEHPNARKYKGANKKGLSKGCFGLKLDRIGSMSGLGC

SEQ ID NO: 3 - protein, 37 aa, Artificial Sequence
  Synthetic Polypeptide
QEHPNARKYKGANKKGLSKGCFGLKLDRIGSMSGLGC

SEQ ID NO: 4 - protein, 34 aa, Artificial Sequence
  Synthetic Polypeptide
PNARKYKGANKKGLSKGCFGLKLDRIGSMSGLGC

SEQ ID NO: 5 - protein, 39 aa, Artificial Sequence
  Synthetic Polypeptide
PGQEHPQARRYRGAQRRGLSRGCFGLKLDRIGSMSGLGC

SEQ ID NO: 6 - protein, 39 aa, Artificial Sequence
  Synthetic Polypeptide
PGQEHPNARRYRGANRRGLSRGCFGLKLDRIGSMSGLGC

SEQ ID NO: 7 - protein, 39 aa, Artificial Sequence
  Synthetic Polypeptide
PGQEHPQARKYKGAQKKGLSKGCFGLKLDRIGSMSGLGC

SEQ ID NO: 8 - protein, 39 aa, Artificial Sequence; identical to SEQ ID NO: 5
  Synthetic Polypeptide
  MISC_FEATURE (1)..(1): N -terminal Acetyl
  MISC_FEATURE (39)..(39): C -terminal OH

SEQ ID NO: 9 - protein, 39 aa, Artificial Sequence; identical to SEQ ID NO: 1
  Synthetic Polypeptide
  MISC_FEATURE (1)..(1): N -terminal Acetyl
  MISC_FEATURE (39)..(39): C -terminal NH2

SEQ ID NO: 10 - protein, 39 aa, Artificial Sequence; identical to SEQ ID NO: 6
  Synthetic Polypeptide
  MISC_FEATURE (1)..(1): N -terminal Acetyl
  MISC_FEATURE (39)..(39): C -terminal OH

SEQ ID NO: 11 - protein, 39 aa, Artificial Sequence; identical to SEQ ID NO: 6
  Synthetic Polypeptide
  MISC_FEATURE (1)..(1): N -terminal Acetyl
  MISC_FEATURE (39)..(39): C -terminal NH2

SEQ ID NO: 12 - protein, 39 aa, Artificial Sequence; identical to SEQ ID NO: 5
  Synthetic Polypeptide
  MISC_FEATURE (1)..(1): N -terminal Acetyl
  MISC_FEATURE (39)..(39): C -terminal NH2

SEQ ID NO: 13 - protein, 39 aa, Artificial Sequence; identical to SEQ ID NO: 7
  Synthetic Polypeptide
  MISC_FEATURE (1)..(1): N -terminal Acetyl
  MISC_FEATURE (39)..(39): C -terminal NH2

SEQ ID NO: 14 - protein, 39 aa, Artificial Sequence; identical to SEQ ID NO: 7
  Synthetic Polypeptide
  MISC_FEATURE (1)..(1): N -terminal Acetyl
  MISC_FEATURE (39)..(39): C -terminal OH

SEQ ID NO: 15 - protein, 52 aa, Artificial Sequence
  Synthetic Polypeptide
LRVDTKSRAAWARLLQEHPNARKYKGANKKGLSKGCFGLKLDRIGSMSGLGC

SEQ ID NO: 16 - protein, 51 aa, Artificial Sequence
  Synthetic Polypeptide
RVDTKSRAAWARLLQEHPNARKYKGANKKGLSKGCFGLKLDRIGSMSGLGC

SEQ ID NO: 17 - protein, 50 aa, Artificial Sequence
  Synthetic Polypeptide
VDTKSRAAWARLLQEHPNARKYKGANKKGLSKGCFGLKLDRIGSMSGLGC

SEQ ID NO: 18 - protein, 49 aa, Artificial Sequence
  Synthetic Polypeptide
DTKSRAAWARLLQEHPNARKYKGANKKGLSKGCFGLKLDRIGSMSGLGC

SEQ ID NO: 19 - protein, 48 aa, Artificial Sequence
  Synthetic Polypeptide
TKSRAAWARLLQEHPNARKYKGANKKGLSKGCFGLKLDRIGSMSGLGC

SEQ ID NO: 20 - protein, 47 aa, Artificial Sequence
  Synthetic Polypeptide
KSRAAWARLLQEHPNARKYKGANKKGLSKGCFGLKLDRIGSMSGLGC

SEQ ID NO: 21 - protein, 46 aa, Artificial Sequence
  Synthetic Polypeptide
SRAAWARLLQEHPNARKYKGANKKGLSKGCFGLKLDRIGSMSGLGC

SEQ ID NO: 22 - protein, 45 aa, Artificial Sequence
  Synthetic Polypeptide
RAAWARLLQEHPNARKYKGANKKGLSKGCFGLKLDRIGSMSGLGC

SEQ ID NO: 23 - protein, 44 aa, Artificial Sequence
  Synthetic Polypeptide
AAWARLLQEHPNARKYKGANKKGLSKGCFGLKLDRIGSMSGLGC

SEQ ID NO: 24 - protein, 43 aa, Artificial Sequence
  Synthetic Polypeptide
AWARLLQEHPNARKYKGANKKGLSKGCFGLKLDRIGSMSGLGC

SEQ ID NO: 25 - protein, 42 aa, Artificial Sequence
  Synthetic Polypeptide
WARLLQEHPNARKYKGANKKGLSKGCFGLKLDRIGSMSGLGC

SEQ ID NO: 26 - protein, 41 aa, Artificial Sequence
  Synthetic Polypeptide
ARLLQEHPNARKYKGANKKGLSKGCFGLKLDRIGSMSGLGC

SEQ ID NO: 27 - protein, 40 aa, Artificial Sequence
  Synthetic Polypeptide
RLLQEHPNARKYKGANKKGLSKGCFGLKLDRIGSMSGLGC

SEQ ID NO: 28 - protein, 39 aa, Artificial Sequence
  Synthetic Polypeptide
LLQEHPNARKYKGANKKGLSKGCFGLKLDRIGSMSGLGC

SEQ ID NO: 29 - protein, 36 aa, Artificial Sequence
  Synthetic Polypeptide
EHPNARKYKGANKKGLSKGCFGLKLDRIGSMSGLGC

SEQ ID NO: 30 - protein, 35 aa, Artificial Sequence
  Synthetic Polypeptide
HPNARKYKGANKKGLSKGCFGLKLDRIGSMSGLGC

SEQ ID NO: 31 - protein, 33 aa, Artificial Sequence
  Synthetic Polypeptide
NARKYKGANKKGLSKGCFGLKLDRIGSMSGLGC

SEQ ID NO: 32 - protein, 32 aa, Artificial Sequence
  Synthetic Polypeptide
ARKYKGANKKGLSKGCFGLKLDRIGSMSGLGC

SEQ ID NO: 33 - protein, 31 aa, Artificial Sequence
  Synthetic Polypeptide
RKYKGANKKGLSKGCFGLKLDRIGSMSGLGC

SEQ ID NO: 34 - protein, 30 aa, Artificial Sequence
  Synthetic Polypeptide
KYKGANKKGLSKGCFGLKLDRIGSMSGLGC

SEQ ID NO: 35 - protein, 29 aa, Artificial Sequence
  Synthetic Polypeptide
YKGANKKGLSKGCFGLKLDRIGSMSGLGC

SEQ ID NO: 36 - protein, 28 aa, Artificial Sequence
  Synthetic Polypeptide
KGANKKGLSKGCFGLKLDRIGSMSGLGC

SEQ ID NO: 37 - protein, 27 aa, Artificial Sequence
  Synthetic Polypeptide
GANKKGLSKGCFGLKLDRIGSMSGLGC

SEQ ID NO: 38 - protein, 26 aa, Artificial Sequence
  Synthetic Polypeptide
ANKKGLSKGCFGLKLDRIGSMSGLGC

SEQ ID NO: 39 - protein, 25 aa, Artificial Sequence
  Synthetic Polypeptide
NKKGLSKGCFGLKLDRIGSMSGLGC

SEQ ID NO: 40 - protein, 24 aa, Artificial Sequence
  Synthetic Polypeptide
KKGLSKGCFGLKLDRIGSMSGLGC

SEQ ID NO: 41 - protein, 23 aa, Artificial Sequence
  Synthetic Polypeptide
KGLSKGCFGLKLDRIGSMSGLGC

SEQ ID NO: 42 - protein, 21 aa, Artificial Sequence
  Synthetic Polypeptide
LSKGCFGLKLDRIGSMSGLGC

SEQ ID NO: 43 - protein, 20 aa, Artificial Sequence
  Synthetic Polypeptide
SKGCFGLKLDRIGSMSGLGC

SEQ ID NO: 44 - protein, 19 aa, Artificial Sequence
  Synthetic Polypeptide
KGCFGLKLDRIGSMSGLGC

SEQ ID NO: 45 - protein, 18 aa, Artificial Sequence
  Synthetic Polypeptide
GCFGLKLDRIGSMSGLGC

SEQ ID NO: 46 - protein, 37 aa, Artificial Sequence
  Synthetic Polypeptide
QEHPNARKYKGANKKGLSKGCFGLKLDRIGSNSGLGC

SEQ ID NO: 47 - protein, 38 aa, Artificial Sequence
  Synthetic Polypeptide
MQEHPNARKYKGANKKGLSKGCFGLKLDRIGSMSGLGC

SEQ ID NO: 48 - protein, 38 aa, Artificial Sequence
  Synthetic Polypeptide
PQEHPNARKYKGANKKGLSKGCFGLKLDRIGSMSGLGC

SEQ ID NO: 49 - protein, 38 aa, Artificial Sequence
  Synthetic Polypeptide
GQEHPNARKYKGANKKGLSKGCFGLKLDRIGSNSGLGC

SEQ ID NO: 50 - protein, 39 aa, Artificial Sequence
  Synthetic Polypeptide
MGQEHPNARKYKGANKKGLSKGCFGLKLDRIGSMSGLGC

SEQ ID NO: 51 - protein, 38 aa, Artificial Sequence
  Synthetic Polypeptide
GQEHPNARKYKGANKKGLSKGCFGLKLDRIGSMSGLGC

SEQ ID NO: 52 - protein, 38 aa, Artificial Sequence
  Synthetic Polypeptide
GQEHPNARKYKGANPKGLSKGCFGLKLDRIGSMSGLGC

SEQ ID NO: 53 - protein, 38 aa, Artificial Sequence
  Synthetic Polypeptide
GQEHPNARKYKGANQKGLSKGCFGLKLDRIGSMSGLGC

SEQ ID NO: 54 - protein, 38 aa, Artificial Sequence
  Synthetic Polypeptide
GQEHPNARKYKGANQQGLSKGCFGLKLDRIGSMSGLGC

SEQ ID NO: 55 - protein, 38 aa, Artificial Sequence
  Synthetic Polypeptide
GQEHPNARKYKGANKPGLSKGCFGLKLDRIGSMSGLGC

SEQ ID NO: 56 - protein, 53 aa, Artificial Sequence
  Synthetic Polypeptide
DLRVDTKSRAAWARLLQEHPNARKYKGANKKGLSKGCFGLKLDRIGSMSGLGC

SEQ ID NO: 57 - DNA, 667 bp, Artificial Sequence
  Synthetic Polynucleotide
atggcactgccatccctgctactggtggtggcagccctggcaggtggggtgcgtcctccgggggcacggaacctgacgctggcggtggtgctgccagaacacaacctgagctatgcctgggcctggccacgggtgggtcctgctgtggcactggctgtggaggcgctgggccgggcactgcccgtggacctgcggtttgtcagctccgaactagacggcgcctgctctgagtacctggcaccactgcgcgctgtggatctcaagctgtaccatgaccccgaccttctgttgggccctggttgtgtgtaccctgctgcctctgtggctcgctttgcctcgcactggcaccttcccctcctgactgcgggtgcagtggcctctggctttgcagctaagaatgagcattatcgtaccctggttcgcactggcccctctgcgcccaagctgggtgagttcgtagtgacattacacgggcacttcaattggactgctcgggctgctttgctgtatctggatgctcgcacagatgaccggccccactacttcaccatcgagggggtgtttgaggccctgcagggcagcaacctcagtgtgcaacaccaggtgtatacccgagagccaggtggccctgagcaagccacccacttcatcagagccaacgggcgca

SEQ ID NO: 58 - DNA, 667 bp, Artificial Sequence; identical to SEQ ID NO: 57
  Synthetic Polynucleotide

SEQ ID NO: 59 - DNA, 669 bp, Artificial Sequence
  Synthetic Polynucleotide
atggcactgccatccctgctactggtggtggcagccctggcaggtggggtgcgtcctccgggggcacggaacctgacgctggcggtggtgctgccagaacacaacctgagctatgcctgggcctggccacgggtgggtcctgctgtggcactggctgtggaggcgctgggccgggcactgcccgtggacctgcggtttgtcagctccgaactagacggcgcctgctctgagtacctggcaccactgcgcgctgtggatctcaagctgtaccatgaccccgaccttctgttgggccctggttgtgtgtaccctgctgcctctgtggctcgctttgcctcgcactggcaccttcccctcctgactgcgggtgcagtggcctctggctttgcagctaagaatgagcattatcgtaccctggttcgcactggcccctctgcgcccaagctgggtgagttcgtagtgacattacacgggcacttcacaattggactgctcgggctgctttgctgtatctggatgctcgcacagatgaccggccccactacttcaccatcgagggggtgtttgaggccctgcagggcagcaacctcagtgtgcaacaccaggtgtatacccgagagccaggtggccctgagcaagccacccacttcatcagagccaacgggcgca

SEQ ID NO: 60 - DNA, 668 bp, Artificial Sequence
  Synthetic Polynucleotide
atggcactgccatccctgctactggtggtggcagccctggcaggtggggtgcgtcctccgggggcacggaacctgacgctggcggtggtgctgccagaacacaacctgagctatgcctgggcctggccacgggtgggtcctgctgtggcactggctgtggaggcgctgggccgggcactgcccgtggacctgcggtttgtcagctccgaactagacggcgcctgctctgagtacctggcaccactgcgcgctgtggatctcaagctgtaccatgaccccgaccttctgttgggccctggttgtgtgtaccctgctgcctctgtggctcgctttgcctcgcactggcaccttcccctcctgactgcgggtgcagtggcctctggctttgcagctaagaatgagcattatcgtaccctggttcgcactggcccctctgcgcccaagctgggtgagttcgtagtgacattacacgggcacttcaattggactgctcgggctgctttgctgtatctggatgctcgcacagatgaccggccccactacttcaccatccgagggggtgtttgaggccctgcagggcagcaacctcagtgtgcaacaccaggtgtatacccgagagccaggtggccctgagcaagccacccacttcatcagagccaacgggcgca

SEQ ID NO: 61 - DNA, 354 bp, Artificial Sequence
  Synthetic Polynucleotide
atggcactgccatccctgctactggtggtggcagccctggcaggtggggtgcgtcctccgggggcacggaacctgacgctggcggtggtgctgccagaacacaacctgagctatgcctgggcctggccacgggtgggtcctgctgtggcactggctgtggaggcgctgggccgggcactgcccgtggacctgcggtttgtcagctccgaactagacggcgcctgctctgagtacctggcaccggggtgtttgaggccctgcagggcagcaacctcagtgtgcaacaccaggtgtatacccgagagccaggtggccctgagcaagccacccacttcatcagagccaacgggcgca

SEQ ID NO: 62 - protein, 1047 aa, Artificial Sequence
  Synthetic Polypeptide
MALPSLLLVVAALAGGVRPPGARNLTLAVVLPEHNLSYAWAWPRVGPAVALAVEALGRALPVDLRFVSSELDGACSEYLAPLRAVDLKLYHDPDLLLGPGCVYPAASVARFASHWHLPLLTAGAVASGFAAKNEHYRTLVRTGPSAPKLGEFVVTLHGHFNWTARAALLYLDARTDDRPHYFTIEGVFEALQGSNLSVQHQVYTREPGGPEQATHFIRANGRIVYICGPLEMLHEILLQAQRENLTNGDYVFFYLDVFGESLRAGPTRATGRPWQDNRTQEQAQALREAFQTVLVITYREPPNPEYQEFQNRLLIRAREDFGVELAPSLMNLIAGCFYDGILLYAQVLNETIQEGGTREDGLRIVEKMQGRRYHGVTGLVVMDKNNDRETDFVLWAMGDLESGDFQPAAHYSGAEKQIWWTGRPIPWVKGAPPLDNPPCAFDLDDPSCDKTPLSTLAIVALGTGITFIMFGVSSFLIFRKLMLEKELASMLWRIRWEELQFGNSDRYHKGAGSRLTLSLRGSSYGSLMTAHGKYQIFANTGHFKGNVVAIKHVNKKRIELTRQVLFELKHMRDVQFNHLTRFIGACIDPPNICIVTEYCPRGSLQDILENDSINLDWMFRYSLINDLVKGMAFLHNSIISSHGSLKSSNCVVDSRFVLKITDYGLASFRSTAEPDDSHALYAKKLWTAPELLSGNPLPTTGMQKADVYSFAIILQEIALRSGPFYLEGLDLSPKEIVQKVRNGQRPYFRPSIDRTQLNEELVLLMERCWAQDPTERPDFGQIKGFIRRFNKEGGTSILDNLLLRMEQYANNLEKLVEERTQAYLEEKRKAEALLYQILPHSVAEQLKRGETVQAEAFDSVTIYFSDIVGFTALSAESTPMQVVTLLNDLYTCFDAIIDNFDVYKVETIGDAYMVVSGLPGRNGQRHAPEIARMALALLDAVSSFRIRHRPHDQLRLRIGVHTGPVCAGVVGLKMPRYCLFGDTVNTASRMESNGQALKIHVSSTTKDALDELGCFQLELRGDVEMKGKGKMRTYWLLGERKGPPGLL

SEQ ID NO: 63 - protein, 1047 aa, Artificial Sequence; identical to SEQ ID NO: 62
  Synthetic Polypeptide

SEQ ID NO: 64 - protein, 245 aa, Artificial Sequence
  Synthetic Polypeptide
MALPSLLLVVAALAGGVRPPGARNLTLAVVLPEHNLSYAWAWPRVGPAVALAVEALGRALPVDLRFVSSELDGACSEYLAPLRAVDLKLYHDPDLLLGPGCVYPAASVARFASHWHLPLLTAGAVASGFAAKNEHYRTLVRTGPSAPKLGEFVVTLHGHFTIGLLGLLCCIWMLAQMTGPTTSPSRGCLRPCRAATSVCNTRCIPESQVALSKPPTSSEPTGALCISAARWRCFMRSCFRPRGRT

SEQ ID NO: 65 - protein, 188 aa, Artificial Seuqence
  Synthetic Polypeptide
MALPSLLLVVAALAGGVRPPGARNLTLAVVLPEHNLSYAWAWPRVGPAVALAVEALGRALPVDLRFVSSELDGACSEYLAPLRAVDLKLYHDPDLLLGPGCVYPAASVARFASHWHLPLLTAGAVASGFAAKNEHYRTLVRTGPSAPKLGEFVVTLHGHFNWTARAALLYLDARTDDRPHYFTIRGGV

SEQ ID NO: 66 - protein, 140 aa, Artificial Sequence
  Synthetic Polypeptide
MALPSLLLVVAALAGGVRPPGARNLTLAVVLPEHNLSYAWAWPRVGPAVALAVEALGRALPVDLRFVSSELDGACSEYLAPGCLRPCRAATSVCNTRCIPESQVALSKPPTSSEPTGALCISAARWRCFMRSCFRPRGRT

SEQ ID NO: 67 - protein, 17 aa, Artificial Sequence
  Synthetic Polypeptide
CFGLKLDRIGSMSGLGC

SEQ ID NO: 68 - protein, 22 aa, Artificial Sequence
  Synthetic Polypeptide
GLSKGCFGLKLDRIGSMSGLGC